European Patent Application EP 4 534 548 A1, published April 9, 2025. Title: Virus-like particles with enhanced optical properties. Applicant: Eberhard Karls Universität Tübingen - Medizinische Fakultät. Application EP. The sequence listing filed with the application follows.

SEQUENCE LISTING (10 sequences)

SEQ ID NO: 1 - protein, 10 aa, synthetic construct
RVTRNYDVHH

SEQ ID NO: 2 - protein, 384 aa, synthetic construct
MAPKRKSGVSKCETKCTKACPRPAPVPKLLIKGGMEVLDLVTGPDSVTEIEAFLNPRMGQPPTPESLTEGGQYYGWSRGINLATSDTEDSPGNNTLPTWSMAKLQLPMLNEDLTCDTLQMWEAVSVKTEVVGSGSLLDVHGFNKPTDTVNTKGISTPVEGSQYHVFAVGGEPLDLQGLVTDARTKYKEEGVVTIKTITKKDMVNKDQVLNPISKAKLDKDGMYPVEIWHPDPAKNENTRYFGNYTGGTTTPPVLQFTNTLTTVLLDENGVGPLCKGEGLYLSCVDIMGWRVTRNYDVHHWRGLPRYFKITLRKRWVKNPYPMASLISSLFNNMLPQVQGQPMEGENTQVEEVRVYDGTEPVPGDPDMTRYVDRFGKTKTVFPGN

SEQ ID NO: 3 - protein, 239 aa, synthetic construct
MGSKGEELFTGVVPILVELDGDVNGHKFSVRGEGEGDATNGKLTLKFICTTGKLPVPWPTLVTTLTYGVQCFSRYPDHMKQHDFFKSAMPEGYVQERTISFKDDGTYKTRAEVKFEGDTLVNRIELKGIDFKEDGNILGHKLEYNFNSHNVYITADKQKNGIKANFKIRHNVEDGSVQLADHYQQNTPIGDGPVLLPDNHYLSTQSVLSKDPNEKRDHMVLLEFVTAAGITHGMDELYK

SEQ ID NO: 4 - protein, 6 aa, synthetic construct
GSGSSH

SEQ ID NO: 5 - protein, 7 aa, synthetic construct
GSSGSGS

SEQ ID NO: 6 - protein, 636 aa, synthetic construct
MAPKRKSGVSKCETKCTKACPRPAPVPKLLIKGGMEVLDLVTGPDSVTEIEAFLNPRMGQPPTPESLTEGGQYYGWSRGINLATSDTEDSPGNNTLPTWSMAKLQLPMLNEDLTCDTLQMWEAVSVKTEVVGSGSLLDVHGFNKPTDTVNTKGISTPVEGSQYHVFAVGGEPLDLQGLVTDARTKYKEEGVVTIKTITKKDMVNKDQVLNPISKAKLDKDGMYPVEIWHPDPAKNENTRYFGNYTGGTTTPPVLQFTNTLTTVLLDENGVGPLCKGEGLYLSCVDIMGWRVTRNGSGSSHMGSKGEELFTGVVPILVELDGDVNGHKFSVRGEGEGDATNGKLTLKFICTTGKLPVPWPTLVTTLTYGVQCFSRYPDHMKQHDFFKSAMPEGYVQERTISFKDDGTYKTRAEVKFEGDTLVNRIELKGIDFKEDGNILGHKLEYNFNSHNVYITADKQKNGIKANFKIRHNVEDGSVQLADHYQQNTPIGDGPVLLPDNHYLSTQSVLSKDPNEKRDHMVLLEFVTAAGITHGMDELYKGSSGSGSYDVHHWRGLPRYFKITLRKRWVKNPYPMASLISSLFNNMLPQVQGQPMEGENTQVEEVRVYDGTEPVPGDPDMTRYVDRFGKTKTVFPGN

SEQ ID NO: 7 - DNA, 39 bp, synthetic construct
  source 1..39: mol_type = other DNA
ggatccagcggttctggaagctatgatgtccatcactgg

SEQ ID NO: 8 - DNA, 40 bp, synthetic construct
  source 1..40: mol_type = other DNA
catatgcgatgagccactgccgtttcttgtaactctccag

SEQ ID NO: 9 - DNA, 45 bp, synthetic construct
  source 1..45: mol_type = other DNA
ggcagtggctcatcgcatatgggtagtaaaggcgaagagctgttc

SEQ ID NO: 10 - DNA, 42 bp, synthetic construct
  source 1..42: mol_type = other DNA
gcttccagaaccgctggatcctttatacagctcgtccatccc